European Patent Application EP 4 321 171 A2, published February 14, 2024. Title: SIRP ALPHA-ANTIBODY FUSION PROTEINS. Applicant: The Board of Trustees of the Leland Stanford Junior University. The sequence listing filed with the application follows.

SEQUENCE LISTING (21 sequences)

SEQ ID NO: 1 - protein, 119 aa, Homo sapiens
EEELQVIQPDKSVLVAAGETATLRCTATSLIPVGPIQWFRGAGPGRELIYNQKEGHFPRVTTVSDLTKRNNMDFSIRIGNITPADAGTYYCVKFRKGSPDDVEFKSGAGTELSVRAKPS

SEQ ID NO: 2 - protein, 5 aa, Homo sapiens
GGGGS

SEQ ID NO: 3 - protein, 13 aa, Homo sapiens
ASTKGPSVFPLAP

SEQ ID NO: 4 - DNA, 708 bp, Homo sapiens
  source 1..708: mol_type = unassigned DNA
  CDS 1..708: protein_id = 16; translation = MDFQVQIISFLLISASVIMSRGQIVLSQSPAILSASPGEKVTMTCRASSSVSYIHWFQQKPGSSPKPWIYATSNLASGVPVRFSGSGSGTSYSLTISRVEAEDAATYYCQQWTSNPPTFGGGTKLEIKRTVAAPSVFIFPPSDEQLKSGTASVVCLLNNFYPREAKVQWKVDNALQSGNSQESVTEQDSKDSTYSLSSTLTLSKADYEKHKVYACEVTHQGLSSPVTKSFNRGEC
atggattttcaggtgcagattatcagcttcctgctaatcagtgcttcagtcataatgtccagaggacaaattgttctctcccagtctccagcaatcctgtctgcatctccaggggagaaggtcacaatgacttgcagggccagctcaagtgtaagttacatccactggttccagcagaagccaggatcctcccccaaaccctggatttatgccacatccaacctggcttctggagtccctgttcgcttcagtggcagtgggtctgggacttcttactctctcaccatcagcagagtggaggctgaagatgctgccacttattactgccagcagtggactagtaacccacccacgttcggaggggggaccaagctggaaatcaaacgtacggtggcggcgccatctgtcttcatcttcccgccatctgatgagcagttgaaatctggaactgcctctgttgtgtgcctgctgaataacttctatcccagagaggccaaagtacagtggaaggtggataacgccctccaatcgggtaactcccaggagagtgtcacagagcaggacagcaaggacagcacctacagcctcagcagcaccctgacgctgagcaaagcagactacgagaaacacaaagtctacgcctgcgaagtcacccatcagggcctgagctcgcccgtcacaaagagcttcaacaggggagagtgttag

SEQ ID NO: 5 - protein, 235 aa, Homo sapiens
MDFQVQIISFLLISASVIMSRGQIVLSQSPAILSASPGEKVTMTCRASSSVSYIHWFQQKPGSSPKPWIYATSNLASGVPVRFSGSGSGTSYSLTISRVEAEDAATYYCQQWTSNPPTFGGGTKLEIKRTVAAPSVFIFPPSDEQLKSGTASVVCLLNNFYPREAKVQWKVDNALQSGNSQESVTEQDSKDSTYSLSSTLTLSKADYEKHKVYACEVTHQGLSSPVTKSFNRGEC

SEQ ID NO: 6 - DNA, 1800 bp, Homo sapiens
  source 1..1800: mol_type = unassigned DNA
  CDS 1..1800: protein_id = 17; translation = MGWSLILLFLVAVATRVLSQVQLQQPGAELVKPGASVKMSCKASGYTFTSYNMHWVKQTPGRGLEWIGAIYPGNGDTSYNQKFKGKATLTADKSSSTAYMQLSSLTSEDSAVYYCARSTYYGGDWYFNVWGAGTTVTVSAASTKGPSVFPLAPSSKSTSGGTAALGCLVKDYFPEPVTVSWNSGALTSGVHTFPAVLQSSGLYSLSSVVTVPSSSLGTQTYICNVNHKPSNTKVDKKVEPKSCDKTHTCPPCPAPELLGGPSVFLFPPKPKDTLMISRTPEVTCVVVDVSHEDPEVKFNWYVDGVEVHNAKTKPREEQYNSTYRVVSVLTVLHQDWLNGKEYKCKVSNKALPAPIEKTISKAKGQPREPQVYTLPPSRDELTKNQVSLTCLVKGFYPSDIAVEWESNGQPENNYKTTPPVLDSDGSFFLYSKLTVDKSRWQQGNVFSCSVMHEALHNHYTQKSLSLSPGKGGGGSGGGGSEEELQVIQPDKSVLVAAGETATLRCTATSLIPVGPIQWFRGAGPGRELIYNQKEGHFPRVTTVSDLTKRNNMDFSIRIGNITPADAGTYYCVKFRKGSPDDVEFKSGAGTELSVRAKPS
atgggttggagcctcatcttgctcttccttgtcgctgttgctacgcgtgtcctgtcccaggtacaactgcagcagcctggggctgagctggtgaagcctggggcctcagtgaagatgtcctgcaaggcttctggctacacatttaccagttacaatatgcactgggtaaaacagacacctggtcggggcctggaatggattggagctatttatcccggaaatggtgatacttcctacaatcagaagttcaaaggcaaggccacattgactgcagacaaatcctccagcacagcctacatgcagctcagcagcctgacatctgaggactctgcggtctattactgtgcaagatcgacttactacggcggtgactggtacttcaatgtctggggcgcagggaccacggtcaccgtctctgcagcgagcaccaagggcccatcggtcttccccctggcaccctcctccaagagcacctctgggggcacagcggccctgggctgcctggtcaaggactacttccccgaaccggtgacggtgtcgtggaactcaggcgccctgaccagcggcgtgcacaccttcccggctgtcctacagtcctcaggactctactccctcagcagcgtggtgaccgtgccctccagcagcttgggcacccagacctacatctgcaacgtgaatcacaagcccagcaacaccaaggtggacaagaaagttgagcccaaatcttgtgacaaaactcacacatgcccaccgtgcccagcacctgaactcctggggggaccgtcagtcttcctcttccccccaaaacccaaggacaccctcatgatctcccggacccctgaggtcacatgcgtggtggtggacgtgagccacgaagaccctgaggtcaagttcaactggtacgtggacggcgtggaggtgcataatgccaagacaaagccgcgggaggagcagtacaacagcacgtaccgtgtggtcagcgtcctcaccgtcctgcaccaggactggctgaatggcaaggagtacaagtgcaaggtctccaacaaagccctcccagcccccatcgagaaaaccatctccaaagccaaagggcagccccgagaaccacaggtgtacaccctgcccccatcccgggatgagctgaccaagaaccaggtcagcctgacctgcctggtcaaaggcttctatcccagcgacatcgccgtggagtgggagagcaatgggcagccggagaacaactacaagaccacgcctcccgtgctggactccgacggctccttcttcctctacagcaagctcaccgtggacaagagcaggtggcagcaggggaacgtcttctcatgctccgtgatgcatgaggctctgcacaaccactacacgcagaagagcctctccctgtctccgggtaaaggtggcggtggctcgggcggtggtgggtcggaggaggagctgcaggtgattcagcctgacaagtccgtgttggttgcagctggagagacagccactctgcgctgcactgcgacctctctgatccctgtggggcccatccagtggttcagaggagctggaccaggccgggaattaatctacaatcaaaaagaaggccacttcccccgggtaacaactgtttcagacctcacaaagagaaacaacatggacttttccatccgcatcggtaacatcaccccagcagatgccggcacctactactgtgtgaagttccggaaagggagccccgatgacgtggagtttaagtctggagcaggcactgagctgtctgtgcgcgccaaaccctcttga

SEQ ID NO: 7 - protein, 599 aa, Homo sapiens
MGWSLILLFLVAVATRVLSQVQLQQPGAELVKPGASVKMSCKASGYTFTSYNMHWVKQTPGRGLEWIGAIYPGNGDTSYNQKFKGKATLTADKSSSTAYMQLSSLTSEDSAVYYCARSTYYGGDWYFNVWGAGTTVTVSAASTKGPSVFPLAPSSKSTSGGTAALGCLVKDYFPEPVTVSWNSGALTSGVHTFPAVLQSSGLYSLSSVVTVPSSSLGTQTYICNVNHKPSNTKVDKKVEPKSCDKTHTCPPCPAPELLGGPSVFLFPPKPKDTLMISRTPEVTCVVVDVSHEDPEVKFNWYVDGVEVHNAKTKPREEQYNSTYRVVSVLTVLHQDWLNGKEYKCKVSNKALPAPIEKTISKAKGQPREPQVYTLPPSRDELTKNQVSLTCLVKGFYPSDIAVEWESNGQPENNYKTTPPVLDSDGSFFLYSKLTVDKSRWQQGNVFSCSVMHEALHNHYTQKSLSLSPGKGGGGSGGGGSEEELQVIQPDKSVLVAAGETATLRCTATSLIPVGPIQWFRGAGPGRELIYNQKEGHFPRVTTVSDLTKRNNMDFSIRIGNITPADAGTYYCVKFRKGSPDDVEFKSGAGTELSVRAKPS

SEQ ID NO: 8 - DNA, 1803 bp, Homo sapiens
  source 1..1803: mol_type = unassigned DNA
  CDS 1..1803: protein_id = 18; translation = MRAWIFFLLCLAGRALAEEELQVIQPDKSVLVAAGETATLRCTATSLIPVGPIQWFRGAGPGRELIYNQKEGHFPRVTTVSDLTKRNNMDFSIRIGNITPADAGTYYCVKFRKGSPDDVEFKSGAGTELSVRAKPSASTKGPSVFPLAPQVQLQQPGAELVKPGASVKMSCKASGYTFTSYNMHWVKQTPGRGLEWIGAIYPGNGDTSYNQKFKGKATLTADKSSSTAYMQLSSLTSEDSAVYYCARSTYYGGDWYFNVWGAGTTVTVSAASTKGPSVFPLAPSSKSTSGGTAALGCLVKDYFPEPVTVSWNSGALTSGVHTFPAVLQSSGLYSLSSVVTVPSSSLGTQTYICNVNHKPSNTKVDKKVEPKSCDKTHTCPPCPAPELLGGPSVFLFPPKPKDTLMISRTPEVTCVVVDVSHEDPEVKFNWYVDGVEVHNAKTKPREEQYNSTYRVVSVLTVLHQDWLNGKEYKCKVSNKALPAPIEKTISKAKGQPREPQVYTLPPSRDELTKNQVSLTCLVKGFYPSDIAVEWESNGQPENNYKTTPPVLDSDGSFFLYSKLTVDKSRWQQGNVFSCSVMHEALHNHYTQKSLSLSPGK
atgagggcttggatcttctttctgctctgcctggccgggcgcgccttggccgaggaggagctgcaggtgattcagcctgacaagtccgtgttggttgcagctggagagacagccactctgcgctgcactgcgacctctctgatccctgtggggcccatccagtggttcagaggagctggaccaggccgggaattaatctacaatcaaaaagaaggccacttcccccgggtaacaactgtttcagacctcacaaagagaaacaacatggacttttccatccgcatcggtaacatcaccccagcagatgccggcacctactactgtgtgaagttccggaaagggagccccgatgacgtggagtttaagtctggagcaggcactgagctgtctgtgcgcgccaaaccctctgcgagcaccaagggcccatcggtcttccccctggcaccccaggtacaactgcagcagcctggggctgagctggtgaagcctggggcctcagtgaagatgtcctgcaaggcttctggctacacatttaccagttacaatatgcactgggtaaaacagacacctggtcggggcctggaatggattggagctatttatcccggaaatggtgatacttcctacaatcagaagttcaaaggcaaggccacattgactgcagacaaatcctccagcacagcctacatgcagctcagcagcctgacatctgaggactctgcggtctattactgtgcaagatcgacttactacggcggtgactggtacttcaatgtctggggcgcagggaccacggtcaccgtctctgcagctagcaccaagggcccatcggtcttccccctggcaccctcctccaagagcacctctgggggcacagcggccctgggctgcctggtcaaggactacttccccgaaccggtgacggtgtcgtggaactcaggcgccctgaccagcggcgtgcacaccttcccggctgtcctacagtcctcaggactctactccctcagcagcgtggtgaccgtgccctccagcagcttgggcacccagacctacatctgcaacgtgaatcacaagcccagcaacaccaaggtggacaagaaagttgagcccaaatcttgtgacaaaactcacacatgcccaccgtgcccagcacctgaactcctggggggaccgtcagtctttctcttccccccaaaacccaaggacaccctcatgatctcccggacccctgaggtcacatgcgtggtggtggacgtgagccacgaagaccctgaggtcaagttcaactggtacgtggacggcgtggaggtgcataatgccaagacaaagccgcgggaggagcagtacaacagcacgtaccgtgtggtcagcgtcctcaccgtcctgcaccaggactggctgaatggcaaggagtacaagtgcaaggtctccaacaaagccctcccagcccccatcgagaaaaccatctccaaagccaaagggcagccccgagaaccacaggtgtacaccctgcccccatcccgggatgagctgaccaagaaccaggtcagcctgacctgcctggtcaaaggcttctatcccagcgacatcgccgtggagtgggagagcaatgggcagccggagaacaactacaagaccacgcctcccgtgctggactccgacggctccttcttcctctatagcaagctcaccgtggacaagagcaggtggcagcaggggaacgtcttctcatgctccgtgatgcatgaggctctgcacaaccactacacgcagaagagcctctccctgtctccgggtaaatga

SEQ ID NO: 9 - protein, 600 aa, Homo sapiens
MRAWIFFLLCLAGRALAEEELQVIQPDKSVLVAAGETATLRCTATSLIPVGPIQWFRGAGPGRELIYNQKEGHFPRVTTVSDLTKRNNMDFSIRIGNITPADAGTYYCVKFRKGSPDDVEFKSGAGTELSVRAKPSASTKGPSVFPLAPQVQLQQPGAELVKPGASVKMSCKASGYTFTSYNMHWVKQTPGRGLEWIGAIYPGNGDTSYNQKFKGKATLTADKSSSTAYMQLSSLTSEDSAVYYCARSTYYGGDWYFNVWGAGTTVTVSAASTKGPSVFPLAPSSKSTSGGTAALGCLVKDYFPEPVTVSWNSGALTSGVHTFPAVLQSSGLYSLSSVVTVPSSSLGTQTYICNVNHKPSNTKVDKKVEPKSCDKTHTCPPCPAPELLGGPSVFLFPPKPKDTLMISRTPEVTCVVVDVSHEDPEVKFNWYVDGVEVHNAKTKPREEQYNSTYRVVSVLTVLHQDWLNGKEYKCKVSNKALPAPIEKTISKAKGQPREPQVYTLPPSRDELTKNQVSLTCLVKGFYPSDIAVEWESNGQPENNYKTTPPVLDSDGSFFLYSKLTVDKSRWQQGNVFSCSVMHEALHNHYTQKSLSLSPGK

SEQ ID NO: 10 - DNA, 1830 bp, Homo sapiens
  source 1..1830: mol_type = unassigned DNA
  CDS 1..1830: protein_id = 19; translation = MGWSLILLFLVAVATRVLSQVQLQQPGAELVKPGASVKMSCKASGYTFTSYNMHWVKQTPGRGLEWIGAIYPGNGDTSYNQKFKGKATLTADKSSSTAYMQLSSLTSEDSAVYYCARSTYYGGDWYFNVWGAGTTVTVSAASTKGPSVFPLAPSSKSTSGGTAALGCLVKDYFPEPVTVSWNSGALTSGVHTFPAVLQSSGLYSLSSVVTVPSSSLGTQTYICNVNHKPSNTKVDKKVEPKSCDKTHTCPPCPAPELLGGPSVFLFPPKPKDTLMISRTPEVTCVVVDVSHEDPEVKFNWYVDGVEVHNAKTKPREEQYNSTYRVVSVLTVLHQDWLNGKEYKCKVSNKALPAPIEKTISKAKGQPREPQVYTLPPSRDELTKNQVSLTCLVKGFYPSDIAVEWESNGQPENNYKTTPPVLDSDGSFFLYSKLTVDKSRWQQGNVFSCSVMHEALHNHYTQKSLSLSPGKGGGGSGGGGSGGGGSGGGGSEEELQVIQPDKSVLVAAGETATLRCTATSLIPVGPIQWFRGAGPGRELIYNQKEGHFPRVTTVSDLTKRNNMDFSIRIGNITPADAGTYYCVKFRKGSPDDVEFKSGAGTELSVRAKPS
atgggttggagcctcatcttgctcttccttgtcgctgttgctacgcgtgtcctgtcccaggtacaactgcagcagcctggggctgagctggtgaagcctggggcctcagtgaagatgtcctgcaaggcttctggctacacatttaccagttacaatatgcactgggtaaaacagacacctggtcggggcctggaatggattggagctatttatcccggaaatggtgatacttcctacaatcagaagttcaaaggcaaggccacattgactgcagacaaatcctccagcacagcctacatgcagctcagcagcctgacatctgaggactctgcggtctattactgtgcaagatcgacttactacggcggtgactggtacttcaatgtctggggcgcagggaccacggtcaccgtctctgcagcgagcaccaagggcccatcggtcttccccctggcaccctcctccaagagcacctctgggggcacagcggccctgggctgcctggtcaaggactacttccccgaaccggtgacggtgtcgtggaactcaggcgccctgaccagcggcgtgcacaccttcccggctgtcctacagtcctcaggactctactccctcagcagcgtggtgaccgtgccctccagcagcttgggcacccagacctacatctgcaacgtgaatcacaagcccagcaacaccaaggtggacaagaaagttgagcccaaatcttgtgacaaaactcacacatgcccaccgtgcccagcacctgaactcctggggggaccgtcagtctttctcttccccccaaaacccaaggacaccctcatgatctcccggacccctgaggtcacatgcgtggtggtggacgtgagccacgaagaccctgaggtcaagttcaactggtacgtggacggcgtggaggtgcataatgccaagacaaagccgcgggaggagcagtacaacagcacgtaccgtgtggtcagcgtcctcaccgtcctgcaccaggactggctgaatggcaaggagtacaagtgcaaggtctccaacaaagccctcccagcccccatcgagaaaaccatctccaaagccaaagggcagccccgagaaccacaggtgtacaccctgcccccatcccgggatgagctgaccaagaaccaggtcagcctgacctgcctggtcaaaggcttctatcccagcgacatcgccgtggagtgggagagcaatgggcagccggagaacaactacaagaccacgcctcccgtgctggactccgacggctccttcttcctctatagcaagctcaccgtggacaagagcaggtggcagcaggggaacgtcttctcatgctccgtgatgcatgaggctctgcacaaccactacacgcagaagagcctctccctgtctccgggtaaaggtggcggtggctcgggcggtggtgggtcgggtggcggcggatctggcggcggtggttctgaggaggagctgcaggtgattcagcctgacaagtccgtgttggttgcagctggagagacagccactctgcgctgcactgcgacctctctgatccctgtggggcccatccagtggttcagaggagctggaccaggccgggaattaatctacaatcaaaaagaaggccacttcccccgggtaacaactgtttcagacctcacaaagagaaacaacatggacttttccatccgcatcggtaacatcaccccagcagatgccggcacctactactgtgtgaagttccggaaagggagccccgatgacgtggagtttaagtctggagcaggcactgagctgtctgtgcgcgccaaaccctcttga

SEQ ID NO: 11 - protein, 609 aa, Homo sapiens
MGWSLILLFLVAVATRVLSQVQLQQPGAELVKPGASVKMSCKASGYTFTSYNMHWVKQTPGRGLEWIGAIYPGNGDTSYNQKFKGKATLTADKSSSTAYMQLSSLTSEDSAVYYCARSTYYGGDWYFNVWGAGTTVTVSAASTKGPSVFPLAPSSKSTSGGTAALGCLVKDYFPEPVTVSWNSGALTSGVHTFPAVLQSSGLYSLSSVVTVPSSSLGTQTYICNVNHKPSNTKVDKKVEPKSCDKTHTCPPCPAPELLGGPSVFLFPPKPKDTLMISRTPEVTCVVVDVSHEDPEVKFNWYVDGVEVHNAKTKPREEQYNSTYRVVSVLTVLHQDWLNGKEYKCKVSNKALPAPIEKTISKAKGQPREPQVYTLPPSRDELTKNQVSLTCLVKGFYPSDIAVEWESNGQPENNYKTTPPVLDSDGSFFLYSKLTVDKSRWQQGNVFSCSVMHEALHNHYTQKSLSLSPGKGGGGSGGGGSGGGGSGGGGSEEELQVIQPDKSVLVAAGETATLRCTATSLIPVGPIQWFRGAGPGRELIYNQKEGHFPRVTTVSDLTKRNNMDFSIRIGNITPADAGTYYCVKFRKGSPDDVEFKSGAGTELSVRAKPS

SEQ ID NO: 12 - DNA, 711 bp, Homo sapiens
  source 1..711: mol_type = unassigned DNA
  CDS 1..711: protein_id = 20; translation = MRAWIFFLLCLAGRALADIVMTQTPLSLSVTPGQPASISCKSSQSLLDGDGKTYLNWLLQKPGQSPQRLIYLVSKLDSGVPDRFSGSGSGTDFTLKISRVEAEDVGVYYCWQGTHFPRTFGQGTKLEIKRTVAAPSVFIFPPSDEQLKSGTASVVCLLNNFYPREAKVQWKVDNALQSGNSQESVTEQDSKDSTYSLSSTLTLSKADYEKHKVYACEVTHQGLSSPVTKSFNRGEC
atgagggcttggatcttctttctgctctgcctggccgggcgcgccttggccgatattgtgatgacccagactccactctctctgtccgtcacccctggacagccggcctccatctcctgcaagtcaagtcagagcctcttagatggtgatggaaagacatatttgaattggttgctgcagaagccaggccagtctccacagcgcctaatctatctggtgtctaaactggactctggagtgccagataggttcagtggcagcgggtcagggacagatttcacactgaaaatcagccgggtggaggctgaggatgttggggtttattactgctggcaaggtacacattttcctcggacgttcggtcagggcaccaagctggaaatcaaacgtacggtggcggcgccatctgtcttcatcttcccgccatctgatgagcagttgaaatctggaactgcctctgttgtgtgcctgctgaataacttctatcccagagaggccaaagtacagtggaaggtggataacgccctccaatcgggtaactcccaggagagtgtcacagagcaggacagcaaggacagcacctacagcctcagcagcaccctgacgctgagcaaagcagactacgagaaacacaaagtctacgcctgcgaagtcacccatcagggcctgagctcgcccgtcacaaagagcttcaacaggggagagtgttag

SEQ ID NO: 13 - protein, 236 aa, Homo sapiens
MRAWIFFLLCLAGRALADIVMTQTPLSLSVTPGQPASISCKSSQSLLDGDGKTYLNWLLQKPGQSPQRLIYLVSKLDSGVPDRFSGSGSGTDFTLKISRVEAEDVGVYYCWQGTHFPRTFGQGTKLEIKRTVAAPSVFIFPPSDEQLKSGTASVVCLLNNFYPREAKVQWKVDNALQSGNSQESVTEQDSKDSTYSLSSTLTLSKADYEKHKVYACEVTHQGLSSPVTKSFNRGEC

SEQ ID NO: 14 - DNA, 1800 bp, Homo sapiens; identical to SEQ ID NO: 6
  source 1..1800: mol_type = unassigned DNA
  CDS 1..1800: protein_id = 21; translation = MGWSLILLFLVAVATRVLSQVQLQQPGAELVKPGASVKMSCKASGYTFTSYNMHWVKQTPGRGLEWIGAIYPGNGDTSYNQKFKGKATLTADKSSSTAYMQLSSLTSEDSAVYYCARSTYYGGDWYFNVWGAGTTVTVSAASTKGPSVFPLAPSSKSTSGGTAALGCLVKDYFPEPVTVSWNSGALTSGVHTFPAVLQSSGLYSLSSVVTVPSSSLGTQTYICNVNHKPSNTKVDKKVEPKSCDKTHTCPPCPAPELLGGPSVFLFPPKPKDTLMISRTPEVTCVVVDVSHEDPEVKFNWYVDGVEVHNAKTKPREEQYNSTYRVVSVLTVLHQDWLNGKEYKCKVSNKALPAPIEKTISKAKGQPREPQVYTLPPSRDELTKNQVSLTCLVKGFYPSDIAVEWESNGQPENNYKTTPPVLDSDGSFFLYSKLTVDKSRWQQGNVFSCSVMHEALHNHYTQKSLSLSPGKGGGGSGGGGSEEELQVIQPDKSVLVAAGETATLRCTATSLIPVGPIQWFRGAGPGRELIYNQKEGHFPRVTTVSDLTKRNNMDFSIRIGNITPADAGTYYCVKFRKGSPDDVEFKSGAGTELSVRAKPS

SEQ ID NO: 15 - protein, 599 aa, Homo sapiens; identical to SEQ ID NO: 7

SEQ ID NO: 16 - protein, 235 aa, Homo sapiens; identical to SEQ ID NO: 5

SEQ ID NO: 17 - protein, 599 aa, Homo sapiens; identical to SEQ ID NO: 7

SEQ ID NO: 18 - protein, 600 aa, Homo sapiens; identical to SEQ ID NO: 9

SEQ ID NO: 19 - protein, 609 aa, Homo sapiens; identical to SEQ ID NO: 11

SEQ ID NO: 20 - protein, 236 aa, Homo sapiens; identical to SEQ ID NO: 13

SEQ ID NO: 21 - protein, 599 aa, Homo sapiens; identical to SEQ ID NO: 7